European Patent Specification EP 4 107 252 B1, published February 19, 2025. Title: Method for the Production of AAV. Applicant: CEVEC Pharmaceuticals GmbH. The sequence listing filed with the application follows.

SEQUENCE LISTING (6 sequences)

SEQ ID NO: 1 - DNA, 25 bp, Artificial sequence
  Primer
agcaatagcatcacaaatttcacaa

SEQ ID NO: 2 - DNA, 29 bp, Artificial sequence
  Primer
ccagacatgataagatacattgatgagtt

SEQ ID NO: 3 - DNA, 36 bp, Artificial sequence
  Probe
agcatttttttcactgcattctagttgtggtttgtc

SEQ ID NO: 4 - DNA, 20 bp, Artificial sequence
  Primer
ttcttcaagtccgccatgcc

SEQ ID NO: 5 - DNA, 20 bp, Artificial sequence
  Primer
aagtcgatgcccttcagctc

SEQ ID NO: 6 - DNA, 34 bp, Artificial sequence
  Probe
cgcaccatcttcttcaaggacgacggcaactaca